European Patent Application EP 4 792 836 A1, published August 19, 2026. Title: 一种多基因纳米载体及其制备方法和应用、一种抗癌药物. Applicant: 天津全和诚生物技术有限公司. The sequence listing filed with the application follows.

SEQUENCE LISTING (26 sequences)

SEQ ID NO: 1 - DNA, 20 bp, synthetic construct
  source 1..20: mol_type = other DNA
cctcccaagatggcccgata

SEQ ID NO: 2 - DNA, 20 bp, synthetic construct
  source 1..20: mol_type = other DNA
cctcctcttccctgtccaaa

SEQ ID NO: 3 - DNA, 48 bp, synthetic construct
  source 1..48: mol_type = other DNA
gtcacacctgctaattcgcggcgggtgtggtggttacgcgcagcgtga

SEQ ID NO: 4 - DNA, 46 bp, synthetic construct
  source 1..46: mol_type = other DNA
gtcacacctgctaatgcttaatgcgccgctacagggcgcgtgggga

SEQ ID NO: 5 - DNA, 45 bp, synthetic construct
  source 1..45: mol_type = other DNA
gtcacacctgctaataagcgcgcgcagcaccatggcctgaaataa

SEQ ID NO: 6 - DNA, 41 bp, synthetic construct
  source 1..41: mol_type = other DNA
gtcacacctgctaatatggtggctttaccaacagtaccgga

SEQ ID NO: 7 - DNA, 42 bp, synthetic construct
  source 1..42: mol_type = other DNA
gtcacacctgctaatccatggcaaagcaaccttctgatgtaa

SEQ ID NO: 8 - DNA, 43 bp, synthetic construct
  source 1..43: mol_type = other DNA
gtcacacctgctaattatcaatgcattctccacaccaggcgga

SEQ ID NO: 9 - DNA, 50 bp, synthetic construct
  source 1..50: mol_type = other DNA
gtcacacctgctaatgataattctagagtcggggcggccggccgcttcga

SEQ ID NO: 10 - DNA, 41 bp, synthetic construct
  source 1..41: mol_type = other DNA
gtcacacctgctaatagcctaccacatttgtagaggtttta

SEQ ID NO: 11 - DNA, 41 bp, synthetic construct
  source 1..41: mol_type = other DNA
gtcacacctgctaatggctccggtgcccgtcagtgggcaga

SEQ ID NO: 12 - DNA, 44 bp, synthetic construct
  source 1..44: mol_type = other DNA
gtcacacctgctaatccgtacgtcacgacacctgaaatggaaga

SEQ ID NO: 13 - DNA, 50 bp, synthetic construct
  source 1..50: mol_type = other DNA
gtcacacctgctaatacggccaccatggactacaaagaccatgacggtga

SEQ ID NO: 14 - DNA, 47 bp, synthetic construct
  source 1..47: mol_type = other DNA
gtcacacctgctaatattctcagacttttgtaatttgtgtatgctga

SEQ ID NO: 15 - DNA, 41 bp, synthetic construct
  source 1..41: mol_type = other DNA
gtcacacctgctaatgaattcgatatcaagcttatcgataa

SEQ ID NO: 16 - DNA, 46 bp, synthetic construct
  source 1..46: mol_type = other DNA
gtcacacctgctaatgcgaaaggacagggaagggagcagtggttca

SEQ ID NO: 17 - DNA, 48 bp, synthetic construct
  source 1..48: mol_type = other DNA
cctcccaagatggcccgatacgatgtacgggccagatatacgcgttga

SEQ ID NO: 18 - DNA, 47 bp, synthetic construct
  source 1..47: mol_type = other DNA
cctcctcttccctgtccaaaaaggacagggaagggagcagtggttca

SEQ ID NO: 19 - DNA, 25 bp, synthetic construct
  source 1..25: mol_type = other DNA
ggcgggtgtggtggttacgcgcagc

SEQ ID NO: 20 - DNA, 25 bp, synthetic construct
  source 1..25: mol_type = other DNA
gcgcttaatgcgccgctacagggcg

SEQ ID NO: 21 - DNA, 45 bp, synthetic construct
  source 1..45: mol_type = other DNA
cgccctgtagcggcgcattaagcgcgagggcctatttcccatgat

SEQ ID NO: 22 - DNA, 45 bp, synthetic construct
  source 1..45: mol_type = other DNA
gctgcgcgtaaccaccacacccgccctcgagaaaaaaggaaacga

SEQ ID NO: 23 - DNA, 40 bp, synthetic construct
  source 1..40: mol_type = other DNA
cctcccaagatggcccgataagctacaacaaggcaaggct

SEQ ID NO: 24 - DNA, 40 bp, synthetic construct
  source 1..40: mol_type = other DNA
cctcctcttccctgtccaaactcgagaaaaaaggaaacga

SEQ ID NO: 25 - DNA, 7000 bp, synthetic construct
  source 1..7000: mol_type = other DNA
cctcccaagatggcccgatacgatgtacgggccagatatacgcgttgacattgattattgactagttattaatagtaatcaattacggggtcattagttcatagcccatatatggagttccgcgttacataacttacggtaaatggcccgcctggctgaccgcccaacgacccccgcccattgacgtcaataatgacgtatgttcccatagtaacgccaatagggactttccattgacgtcaatgggtggagtatttacggtaaactgcccacttggcagtacatcaagtgtatcatatgccaagtacgccccctattgacgtcaatgacggtaaatggcccgcctggcattatgcccagtacatgaccttatgggactttcctacttggcagtacatctacgtattagtcatcgctattaccatggtgatgcggttttggcagtacatcaatgggcgtggatagcggtttgactcacggggatttccaagtctccaccccattgacgtcaatgggagtttgttttggcaccaaaatcaacgggactttccaaaatgtcgtaacaactccgccccattgacgcaaatgggcggtaggcgtgtacggtgggaggtctatataagcagagctctctggctaactagagaacccactgcttactggcttatcgaaattaatacgactcactatagggagacccaagcttaccatggcctacccctacgacgtgcccgactacgcctccctcggatccgaggagccgcagtcagatcctagcgtcgagccccctctgagtcaggaaacattttcagacctatggaaactacttcctgaaaacaacgttctgtcccccttgccgtcccaagcaatggatgatttgatgctgtccccggacgatattgaacaatggttcactgaagacccaggtccagatgaagctcccagaatgccagaggctgctccccccgtggcccctgcaccagcagctcctacaccggcggcccctgcaccagccccctcctggcccctgtcatcttctgtcccttcccagaaaacctaccagggcagctacggtttccgtctgggcttcttgcattctgggacagccaagtctgtgacttgcacgtactcccctgccctcaacaagatgttttgccaactggccaagacctgccctgtgcagctgtgggttgattccacacccccgcccggcacccgcgtccgcgccatggccatctacaagcagtcacagcacatgacggaggttgtgaggcgctgcccccaccatgagcgctgctcagatagcgatggtctggcccctcctcagcatcttatccgagtggaaggaaatttgcgtgtggagtatttggatgacagaaacacttttcgacatagtgtggtggtgccctatgagccgcctgaggttggctcagactgtaccaccatccactacaactacatgtgtaacagttcctgcatgggcggcatgaaccggaggcccatcctcaccatcatcacactggaagactccagtggtaatctactgggacggaacagctttgaggtgcgtgtttgtgcctgtcctgggagagaccggcgcacagaggaagagaatctccgcaagaaaggggagcctcaccacgagctgcccccagggagcactaagcgagcactgcccaacaacaccagctcctctccccagccaaagaagaaaccactggatggagaatatttcacccttcagatccgtgggcgtgagcgcttcgagatgttccgagagctgaatgaggccttggaactcaaggatgcccaggctgggaaggagccaggggggagcagggctcactccagccacctgaagtccaaaaagggtcagtctacctcccgccataaaaaactcatgttcaagacagaagggcctgactcagactgagaattctgcagatatccatcacactggcggccgctcgagcatgcatctagagggccctattctatagtgtcacctaaatgctagagctcgctgatcagcctcgactgtgccttctagttgccagccatctgttgtttgcccctcccccgtgccttccttgaccctggaaggtgccactcccactgtcctttcctaataaaatgaggaaattgcatcgcattgtctgagtaggtgtcattctattctggggggtggggtggggcaggacagcaagggggaggattgggaagacaatagcaggcatgctggggatgcggtgggctctatggcttctgaggcggaaagaaccagctggggctctagggggtatccccacgcgccctgtagcggcgcattaagcgcgcgcagcaccatggcctgaaataacctctgaaagaggaacttggttaggtaccttctgaggcggaaagaaccagctgtggaatgtgtgtcagttagggtgtggaaagtccccaggctccccagcaggcagaagtatgcaaagcatgcatctcaattagtcagcaaccaggtgtggaaagtccccaggctccccagcaggcagaagtatgcaaagcatgcatctcaattagtcagcaaccatagtcccgcccctaactccgcccatcccgcccctaactccgcccagttccgcccattctccgccccatggctgactaattttttttatttatgcagaggccgaggccgcctcggcctctgagctattccagaagtagtgaggaggcttttttggaggcctaggcttttgcaaaaagcttggcaatccggtactgttggtaaagccaccatggcaaagcaaccttctgatgtaagttctgagtgtgaccgagaaggtagacaattgcagcctgcggagaggcctccccagctcagacctggggcccctacctccctacagacagagccacaagcttccatgaggcaggctgaacctgcagatatgcgcccagagatatggatcgcccaagagttgcggcgtattggagacgagtttaacgcttactatgcaaggagggtatttttgaataattaccaagcagccgaagaccacccacgaatggttatcttacgactgttacgttacattgtccgcctggtgtggagaatgcattgataattctagagtcggggcggccggccgcttcgagcagacatgataagatacattgatgagtttggacaaaccacaactagaatgcagtgaaaaaaatgctttatttgtgaaatttgtgatgctattgctttatttgtaaccattataagctgcaataaacaagttaacaacaacaattgcattcattttatgtttcaggttcagggggaggtgtgggaggttttttaaagcaagtaaaacctctacaaatgtggtaggctccggtgcccgtcagtgggcagagcgcacatcgcccacagtccccgagaagttggggggaggggtcggcaattgaaccggtgcctagagaaggtggcgcggggtaaactgggaaagtgatgtcgtgtactggctccgcctttttcccgagggtgggggagaaccgtatataagtgcagtagtcgccgtgaacgttctttttcgcaacgggtttgccgccagaacacaggtaagtgccgtgtgtggttcccgcgggcctggcctctttacgggttatggcccttgcgtgccttgaattacttccacctggctgcagtacgtgattcttgatcccgagcttcgggttggaagtgggtgggagagttcgaggccttgcgcttaaggagccccttcgcctcgtgcttgagttgaggcctggcctgggcgctggggccgccgcgtgcgaatctggtggcaccttcgcgcctgtctcgctgctttcgataagtctctagccatttaaaatttttgatgacctgctgcgacgctttttttctggcaagatagtcttgtaaatgcgggccaagatctgcacactggtatttcggtttttggggccgcgggcggcgacggggcccgtgcgtcccagcgcacatgttcggcgaggcggggcctgcgagcgcggccaccgagaatcggacgggggtagtctcaagctggccggcctgctctggtgcctggcctcgcgccgccgtgtatcgccccgccctgggcggcaaggctggcccggtcggcaccagttgcgtgagcggaaagatggccgcttcccggccctgctgcagggagctcaaaatggaggacgcggcgctcgggagagcgggcgggtgagtcacccacacaaaggaaaagggcctttccgtcctcagccgtcgcttcatgtgactccacggagtaccgggcgccgtccaggcacctcgattagttctcgagcttttggagtacgtcgtctttaggttggggggaggggttttatgcgatggagtttccccacactgagtgggtggagactgaagttaggccagcttggcacttgatgtaattctccttggaatttgccctttttgagtttggatcttggttcattctcaagcctcagacagtggttcaaagtttttttcttccatttcaggtgtcgtgacgtacggccaccatggactacaaagaccatgacggtgattataaagatcatgacatcgactacaaggatgacgatgacaagcttggtaccgagctcggatccatgacagccatcatcaaagagatcgttagcagaaacaaaaggagatatcaagaggatggattcgacttagacttgacctatatttatccaaacattattgctatgggatttcctgcagaaagacttgaaggcgtatacaggaacaatattgatgatgtagtaaggtttttggattcaaagcataaaaaccattacaagatatacaatctttgtgctgaaagacattatgacaccgccaaatttaattgcagagttgcacaatatccttttgaagaccataacccaccacagctagaacttatcaaacccttttgtgaagatcttgaccaatggctaagtgaagatgacaatcatgttgcagcaattcactgtaaagctggaaagggacgaactggtgtaatgatatgtgcatatttattacatcggggcaaatttttaaaggcacaagaggccctagatttctatggggaagtaaggaccagagacaaaaagggagtaactattcccagtcagaggcgctatgtgtattattatagctacctgttaaagaatcatctggattatagaccagtggcactgttgtttcacaagatgatgtttgaaactattccaatgttcagtggcggaacttgcaatcctcagtttgtggtctgccagctaaaggtgaagatatattcctccaattcaggacccacacgacgggaagacaagttcatgtactttgagttccctcagccgttacctgtgtgtggtgatatcaaagtagagttcttccacaaacagaacaagatgctaaaaaaggacaaaatgtttcacttttgggtaaatacattcttcataccaggaccagaggaaacctcagaaaaagtagaaaatggaagtctatgtgatcaagaaatcgatagcatttgcagtatagagcgtgcagataatgacaaggaatatctagtacttactttaacaaaaaatgatcttgacaaagcaaataaagacaaagccaaccgatacttttctccaaattttaaggtgaagctgtacttcacaaaaacagtagaggagccgtcaaatccagaggctagcagttcaacttctgtaacaccagatgttagtgacaatgaacctgatcattatagatattctgacaccactgactctgatccagagaatgaaccttttgatgaagatcagcatacacaaattacaaaagtctgagaattcgatatcaagcttatcgataatcaacctctggattacaaaatttgtgaaagattgactggtattcttaactatgttgctccttttacgctatgtggatacgctgctttaatgcctttgtatcatgctattgcttcccgtatggctttcattttctcctccttgtataaatcctggttgctgtctctttatgaggagttgtggcccgttgtcaggcaacgtggcgtggtgtgcactgtgtttgctgacgcaacccccactggttggggcattgccaccacctgtcagctcctttccggaactttcgctttccccctccctattgccacggcggaactcatcgccgcctgccttgcccgctgctggacaggggctcggctgttgggcactgacaattccgtggtgttgtcggggaaatcatcgtcctttccttggctgctcgcctatgttgccacctggattctgcgcgggacgtccttctgctacgtcccttcggccctcaatccagcggaccttccttcccgcggcctgctgccggctctgcggcctcttccgcgtcttcgccttcgccctcagacgagtcggatctccctttgggccgcctccccgcatcgataccgagcgctgctcgagagatctacgggtggcatccctgtgacccctccccagtgcctctcctggccctggaagttgccactccagtgcccaccagccttgtcctaataaaattaagttgcatcattttgtctgactaggtgtccttctataatattatggggtggaggggggtggtatggagcaaggggcaagttgggaagacaacctgtagggcctgcggggtctattgggaaccaagctggagtgcagtggcacaatcttggctcactgcaatctccgcctcctgggttcaagcgattctcctgcctcagcctcccgagttgttgggattccaggcatgcatgaccaggctcagctaatttttgtttttttggtagagacggggtttcaccatattggccaggctggtctccaactcctaatctcaggtgatctacccaccttggcctcccaaattgctgggattacaggcgtgaaccactgctcccttccctgtcctttttggacagggaagaggagg

SEQ ID NO: 26 - DNA, 2932 bp, synthetic construct
  source 1..2932: mol_type = other DNA
cctcccaagatggcccgataagctacaacaaggcaaggcttgaccgacaattgcatgaagaatctgcttagggttaggcgttttgcgctgcttcgcgatgtacgggccagatatacgcgttgacattgattattgactagttattaatagtaatcaattacggggtcattagttcatagcccatatatggagttccgcgttacataacttacggtaaatggcccgcctggctgaccgcccaacgacccccgcccattgacgtcaataatgacgtatgttcccatagtaacgccaatagggactttccattgacgtcaatgggtggagtatttacggtaaactgcccacttggcagtacatcaagtgtatcatatgccaagtacgccccctattgacgtcaatgacggtaaatggcccgcctggcattatgcccagtacatgaccttatgggactttcctacttggcagtacatctacgtattagtcatcgctattaccatggtgatgcggttttggcagtacatcaatgggcgtggatagcggtttgactcacggggatttccaagtctccaccccattgacgtcaatgggagtttgttttggcaccaaaatcaacgggactttccaaaatgtcgtaacaactccgccccattgacgcaaatgggcggtaggcgtgtacggtgggaggtctatataagcagagctctctggctaactagagaacccactgcttactggcttatcgaaattaatacgactcactatagggagacccaagcttaccatggcctacccctacgacgtgcccgactacgcctccctcggatccgaggagccgcagtcagatcctagcgtcgagccccctctgagtcaggaaacattttcagacctatggaaactacttcctgaaaacaacgttctgtcccccttgccgtcccaagcaatggatgatttgatgctgtccccggacgatattgaacaatggttcactgaagacccaggtccagatgaagctcccagaatgccagaggctgctccccccgtggcccctgcaccagcagctcctacaccggcggcccctgcaccagccccctcctggcccctgtcatcttctgtcccttcccagaaaacctaccagggcagctacggtttccgtctgggcttcttgcattctgggacagccaagtctgtgacttgcacgtactcccctgccctcaacaagatgttttgccaactggccaagacctgccctgtgcagctgtgggttgattccacacccccgcccggcacccgcgtccgcgccatggccatctacaagcagtcacagcacatgacggaggttgtgaggcgctgcccccaccatgagcgctgctcagatagcgatggtctggcccctcctcagcatcttatccgagtggaaggaaatttgcgtgtggagtatttggatgacagaaacacttttcgacatagtgtggtggtgccctatgagccgcctgaggttggctcagactgtaccaccatccactacaactacatgtgtaacagttcctgcatgggcggcatgaaccggaggcccatcctcaccatcatcacactggaagactccagtggtaatctactgggacggaacagctttgaggtgcgtgtttgtgcctgtcctgggagagaccggcgcacagaggaagagaatctccgcaagaaaggggagcctcaccacgagctgcccccagggagcactaagcgagcactgcccaacaacaccagctcctctccccagccaaagaagaaaccactggatggagaatatttcacccttcagatccgtgggcgtgagcgcttcgagatgttccgagagctgaatgaggccttggaactcaaggatgcccaggctgggaaggagccaggggggagcagggctcactccagccacctgaagtccaaaaagggtcagtctacctcccgccataaaaaactcatgttcaagacagaagggcctgactcagactgagaattctgcagatatccatcacactggcggccgctcgagcatgcatctagagggccctattctatagtgtcacctaaatgctagagctcgctgatcagcctcgactgtgccttctagttgccagccatctgttgtttgcccctcccccgtgccttccttgaccctggaaggtgccactcccactgtcctttcctaataaaatgaggaaattgcatcgcattgtctgagtaggtgtcattctattctggggggtggggtggggcaggacagcaagggggaggattgggaagacaatagcaggcatgctggggatgcggtgggctctatggcttctgaggcggaaagaaccagctggggctctagggggtatccccacgcgccctgtagcggcgcattaagcgcgagggcctatttcccatgattccttcatatttgcatatacgatacaaggctgttagagagataattggaattaatttgactgtaaacacaaagatattagtacaaaatacgtgacgtagaaagtaataatttcttgggtagtttgcagttttaaaattatgttttaaaatggactatcatatgcttaccgtaacttgaaagtatttcgatttcttggctttatatatcttgtggaaaggacgaaacaccgcttcaccaacaggaactatgcgaacatagttcctgttggtgaagccacagttcggtaagggagagagaatgtcaagaggcgaacacgaatgttcgcctcttgacattctccacagttcggtaagggagagctcatttctgaagaggacttcgaaaagtcctcttcagaaatgagccacagttcggtaagggagaggaaacgacgagaacagttgacgaatcaactgttctcgtcgtttccttttttctcgagtttggacagggaagaggagg